European Patent Application EP 4 537 834 A1, published April 16, 2025. Title: Precision immunosuppression as prevention and therapy for graft-versus-host disease. Applicant: Eberhard Karls Universität Tübingen - Medizinische Fakultät. Application EP. The sequence listing filed with the application follows.

SEQUENCE LISTING (14 sequences)

SEQ ID NO: 1 - RNA, 21 nt, synthetic construct
  source 1..21: mol_type = other RNA
tagttgtagttacttttggca

SEQ ID NO: 2 - RNA, 16 nt, synthetic construct
  source 1..16: mol_type = other RNA
aaagtaactacaacta

SEQ ID NO: 3 - RNA, 21 nt, synthetic construct
  source 1..21: mol_type = other RNA
ttgtgtagcgttctagattga

SEQ ID NO: 4 - RNA, 16 nt, synthetic construct
  source 1..16: mol_type = other RNA
ctagaacgctacacaa

SEQ ID NO: 5 - RNA, 21 nt, synthetic construct
  source 1..21: mol_type = other RNA
tttagttacattctggtgaga

SEQ ID NO: 6 - RNA, 16 nt, synthetic construct
  source 1..16: mol_type = other RNA
ccagaatgtaactaaa

SEQ ID NO: 7 - RNA, 21 nt, synthetic construct
  source 1..21: mol_type = other RNA
tcttcatttagctttgttaca

SEQ ID NO: 8 - RNA, 16 nt, synthetic construct
  source 1..16: mol_type = other RNA
caaagctaaatgaaga

SEQ ID NO: 9 - RNA, 21 nt, synthetic construct
  source 1..21: mol_type = other RNA
tgcaatacaaatgctacataa

SEQ ID NO: 10 - RNA, 16 nt, synthetic construct
  source 1..16: mol_type = other RNA
tagcatttgtattgca

SEQ ID NO: 11 - RNA, 21 nt, synthetic construct
  source 1..21: mol_type = other RNA
taggtaggaagaatctgctca

SEQ ID NO: 12 - RNA, 16 nt, synthetic construct
  source 1..16: mol_type = other RNA
agattcttcctaccta

SEQ ID NO: 13 - RNA, 21 nt, synthetic construct
  source 1..21: mol_type = other RNA
ttgaccaagaggctgcagaga

SEQ ID NO: 14 - RNA, 16 nt, synthetic construct
  source 1..16: mol_type = other RNA
gcagcctcttggtcaa